European Patent Application EP 4 166 161 A1, published April 19, 2023. Title: COMPOSITIONS AND METHODS TO PROGRAM THERAPEUTIC CELLS USING TARGETED NUCLEIC ACID NANOCARRIERS. Applicant: Fred Hutchinson Cancer Center. Application EP. The sequence listing filed with the application follows.

SEQUENCE LISTING (57 sequences)

SEQ ID NO: 1 - protein, 887 aa, synthetic construct
  REGION 1..887: note = megaTAL protein specific for TCRalpha
MGSCRYPYDVPDYAPPKKKRKVVDLRTLGYSQQQQEKIKPKVRSTVAQHHEALVGHGFTHAHIVALSQHPAALGTVAVTYQHIITALPEATHEDIVGVGKQWSGARALEALLTDAGELRGPPLQLDTGQLVKIAKRGGVTAMEAVHASRNALTGAPLNLTPDQVVAIASNIGGKQALETVQRLLPVLCQDHGLTPDQVVAIASNIGGKQALETVQRLLPVLCQDHGLTPDQVVAIASNIGGKQALETVQRLLPVLCQDHGLTPDQVVAIASNGGGKQALETVQRLLPVLCQDHGLTPDQVVAIASHDGGKQALETVQRLLPVLCQDHGLTPDQVVAIASHDGGKQALETVQRLLPVLCQDHGLTPDQVVAIASNIGGKQALETVQRLLPVLCQDHGLTPDQVVAIASNNGGKQALETVQRLLPVLCQDHGLTPDQVVAIASNGGGKQALETVQRLLPVLCQDHGLTPDQVVAIASNNGGKQALETVQRLLPVLCQDHGLTPDQVVAIASNIGGKQALESIVAQLSRPDPALAALTNDHLVALACLGGRPAMDAVKKGLPHAPELIRRVNRRIGERTSHRVAISRVGGSSRRESINPWILTGFADAEGSFILDIRNRNNESNRYRTSLRFQITLHNKDKSILENIQSTWKVGKITNSGDRAVMLRVTRFEDLKVIIDHFEKYPLITQKLGDYKLFKQAFSVMENKEHLKENGIKELVRIKAKMNWGLTDELKKAFPENISKERPLINKNIPNFKWLAGFTSGDGYFGVNLKKVKGNAKVYVGLRFSISQHIRDKNLMNSLITYLGCGSIWEKNKSEFSWLEFVVTKFSDINDKIIPVFQENTLIGVKLEDFEDWCKVAKLIEEKKHLTESGLDEIKKIKLNMNKGRVF

SEQ ID NO: 2 - DNA, 2464 bp, Homo sapiens
  source 1..2464: mol_type = genomic DNA
actctaaaacgagaagtacaagtgagttcccccaaggggtcggccgcgcctcttcctgtccccgccctgccggctgccccaggccagtggagtggcagccccagaactgggaccaccgggggtggtgaggcggcccggcactgggagctgcatctgaggcttagtccctgagctctctgcctgcccagactagctgcacctcctcattccctgcgcccccttcctctccggaagcccccaggatggtgaggtggtttcaccgagacctcagtgggctggatgcagagaccctgctcaagggccgaggtgtccacggtagcttcctggctcggcccagtcgcaagaaccagggtgacttctcgctctccgtcagggtgggggatcaggtgacccatattcggatccagaactcaggggatttctatgacctgtatggaggggagaagtttgcgactctgacagagctggtggagtactacactcagcagcagggtgtcctgcaggaccgcgacggcaccatcatccacctcaagtacccgctgaactgctccgatcccactagtgagaggtggtaccatggccacatgtctggcgggcaggcagagacgctgctgcaggccaagggcgagccctggacgtttcttgtgcgtgagagcctcagccagcctggagacttcgtgctttctgtgctcagtgaccagcccaaggctggcccaggctccccgctcagggtcacccacatcaaggtcatgtgcgagggtggacgctacacagtgggtggtttggagaccttcgacagcctcacggacctggtggagcatttcaagaagacggggattgaggaggcctcaggcgcctttgtctacctgcggcagccgtactatgccacgagggtgaatgcggctgacattgagaaccgagtgttggaactgaacaagaagcaggagtccgaggatacagccaaggctggcttctgggaggagtttgagagtttgcagaagcaggaggtgaagaacttgcaccagcgtctggaagggcagcggccagagaacaagggcaagaaccgctacaagaacattctcccctttgaccacagccgagtgatcctgcagggacgggacagtaacatccccgggtccgactacatcaatgccaactacatcaagaaccagctgctaggccctgatgagaacgctaagacctacatcgccagccagggctgtctggaggccacggtcaatgacttctggcagatggcgtggcaggagaacagccgtgtcatcgtcatgaccacccgagaggtggagaaaggccggaacaaatgcgtcccatactggcccgaggtgggcatgcagcgtgcttatgggccctactctgtgaccaactgcggggagcatgacacaaccgaatacaaactccgtaccttacaggtctccccgctggacaatggagacctgattcgggagatctggcattaccagtacctgagctggcccgaccatggggtccccagtgagcctgggggtgtcctcagcttcctggaccagatcaaccagcggcaggaaagtctgcctcacgcagggcccatcatcgtgcactgcagcgccggcatcggccgcacaggcaccatcattgtcatcgacatgctcatggagaacatctccaccaagggcctggactgtgacattgacatccagaagaccatccagatggtgcgggcgcagcgctcgggcatggtgcagacggaggcgcagtacaagttcatctacgtggccatcgcccagttcattgaaaccactaagaagaagctggaggtcctgcagtcgcagaagggccaggagtcggagtacgggaacatcacctatcccccagccatgaagaatgcccatgccaaggcctcccgcacctcgtccaagagcttggagtctagtgcagggaccgtggctgcgtcacctgtgagacggggtggccagaggggactgccagtgccgggtccccctgtgctgtctcctgacctgcaccaactgcctgtacttgcccccctgcacccggctgcagacacaaggaggatgtgtatgagaacctgcacactaagaacaagagggaggagaaagtgaagaagcagcggtcagcagacaaggagaagagcaagggttccctcaagaggaagtgagcggtgctgtcctcaggtggccatgcctcagccctgaccctgtggaagcatttcgcgatggacagactcacaacctgaacctaggagtgccccattcttttgtaatttaaatggctgcatcccccccacctctccctgaccctgtatatagcccagccaggccccaggcagggccaacccttctcctcttgtaaataaagccctgggatcactgtgaaaaaaaaaaaaaaaaaaaaaaaaaaaaaaaaaaaaaaaaaaaaaaaaaaaaaaaaaaaaaaaaaaaaaaaaaaa

SEQ ID NO: 3 - DNA, 867 bp, Homo sapiens
  source 1..867: mol_type = genomic DNA
atgcagatcccacaggcgccctggccagtcgtctgggcggtgctacaactgggctggcggccaggatggttcttagactccccagacaggccctggaacccccccaccttctccccagccctgctcgtggtgaccgaaggggacaacgccaccttcacctgcagcttctccaacacatcggagagcttcgtgctaaactggtaccgcatgagccccagcaaccagacggacaagctggccgccttccccgaggaccgcagccagcccggccaggactgccgcttccgtgtcacacaactgcccaacgggcgtgacttccacatgagcgtggtcagggcccggcgcaatgacagcggcacctacctctgtggggccatctccctggcccccaaggcgcagatcaaagagagcctgcgggcagagctcagggtgacagagagaagggcagaagtgcccacagcccaccccagcccctcacccaggccagccggccagttccaaaccctggtggttggtgtcgtgggcggcctgctgggcagcctggtgctgctagtctgggtcctggccgtcatctgctcccgggccgcacgagggacaataggagccaggcgcaccggccagcccctgaaggaggacccctcagccgtgcctgtgttctctgtggactatggggagctggatttccagtggcgagagaagaccccggagccccccgtgccctgtgtccctgagcagacggagtatgccaccattgtctttcctagcggaatgggcacctcatcccccgcccgcaggggctcagctgacggccctcggagtgcccagccactgaggcctgaggatggacactgctcttggcccctctga

SEQ ID NO: 4 - DNA, 420 bp, Homo sapiens
  source 1..420: mol_type = genomic DNA
atgacatccattcgagctgtatttatattcctgtggctgcagctggacttggtgaatggagagaatgtggagcagcatccttcaaccctgagtgtccaggagggagacagcgctgttatcaagtgtacttattcagacagtgcctcaaactacttcccttggtataagcaagaacttggaaaaagacctcagcttattatagacattcgttcaaatgtgggcgaaaagaaagaccaacgaattgctgttacattgaacaagacagccaaacatttctccctgcacatcacagagacccaacctgaagactcggctgtctacttctgtgcagcaagtaggaaggactctgggggttaccagaaagttacctttggaactggaacaaagctccaagtcatcccaaatatccagaaccctgac

SEQ ID NO: 5 - DNA, 1027 bp, Homo sapiens
  source 1..1027: mol_type = genomic DNA
ttggattatcaagtgtcaagtccaatctatgacatcaattattatacatcggagccctgccaaaaaatcaatgtgaagcaaatcgcagcccgcctcctgcctccgctctactcactggtgttcatctttggttttgtgggcaacatgctggtcatcctcatcctgataaactgcaaaaggctgaagagcatgactgacatctacctgctcaacctggccatctctgacctgtttttccttcttactgtccccttctgggctcactatgctgccgcccagtgggactttggaaatacaatgtgtcaactcttgacagggctctattttataggcttcttctctggaatcttcttcatcatcctcctgacaatcgataggtacctggctgtcgtccatgctgtgtttgctttaaaagccaggacggtcacctttggggtggtgacaagtgtgatcacttgggtggtggctgtgtttgcgtctctcccaggaatcatctttaccagatctcaaaaagaaggtcttcattacacctgcagctctcattttccatacattaaagatagtcatcttggggctggtcctgccgctgcttgtcatggtcatctgctactcgggaatcctaaaaactctgcttcggtgtcgaaatgagaagaagaggcacagggctgtgaggcttatcttcaccatcatgattgtttattttctcttctgggctccctacaacattgtccttctcctgaacaccttccaggaattctttggcctgaataattgcagtagctctaacaggttggaccaagctatgcaggtgacagagactcttgggatgacgcactgctgcatcaaccccatcatctatgcctttgtcggggagaagttcagaaactacctcttagtcttcttccaaaagcacattgccaaacgcttctgcaaatgctgttctattttccagcaagaggctcccgagcgagcaagctcagtttacacccgatccactggggagcaggaaatatctgtgggcttgtga

SEQ ID NO: 6 - DNA, 1912 bp, Homo sapiens
  source 1..1912: mol_type = genomic DNA
ttttttttcttccctctagtgggcggggcagaggagttagccaagatgtgactttgaaaccctcagcgtctcagtgcccttttgttctaaacaaagaattttgtaattggttctaccaaagaaggatataatgaagtcactatgggaaaagatggggaggagagttgtaggattctacattaattctcttgtgcccttagcccactacttcagaatttcctgaagaaagcaagcctgaattggttttttaaattgctttaaaaattttttttaactgggttaatgcttgctgaattggaagtgaatgtccattcctttgcctcttttgcagatatacacttcagataactacaccgaggaaatgggctcaggggactatgactccatgaaggaaccctgtttccgtgaagaaaatgctaatttcaataaaatcttcctgcccaccatctactccatcatcttcttaactggcattgtgggcaatggattggtcatcctggtcatgggttaccagaagaaactgagaagcatgacggacaagtacaggctgcacctgtcagtggccgacctcctctttgtcatcacgcttcccttctgggcagttgatgccgtggcaaactggtactttgggaacttcctatgcaaggcagtccatgtcatctacacagtcaacctctacagcagtgtcctcatcctggccttcatcagtctggaccgctacctggccatcgtccacgccaccaacagtcagaggccaaggaagctgttggctgaaaaggtggtctatgttggcgtctggatccctgccctcctgctgactattcccgacttcatctttgccaacgtcagtgaggcagatgacagatatatctgtgaccgcttctaccccaatgacttgtgggtggttgtgttccagtttcagcacatcatggttggccttatcctgcctggtattgtcatcctgtcctgctattgcattatcatctccaagctgtcacactccaagggccaccagaagcgcaaggccctcaagaccacagtcatcctcatcctggctttcttcgcctgttggctgccttactacattgggatcagcatcgactccttcatcctcctggaaatcatcaagcaagggtgtgagtttgagaacactgtgcacaagtggatttccatcaccgaggccctagctttcttccactgttgtctgaaccccatcctctatgctttccttggagccaaatttaaaacctctgcccagcacgcactcacctctgtgagcagagggtccagcctcaagatcctctccaaaggaaagcgaggtggacattcatctgtttccactgagtctgagtcttcaagttttcactccagctaacacagatgtaaaagacttttttttatacgataaataacttttttttaagttacacatttttcagatataaaagactgaccaatattgtacagtttttattgcttgttggatttttgtcttgtgtttctttagtttttgtgaagtttaattgacttatttatataaattttttttgtttcatattgatgtgtgtctaggcaggacctgtggccaagttcttagttgctgtatgtctcgtggtaggactgtagaaaagggaactgaacattccagagcgtgtagtgaatcacgtaaagctagaaatgatccccagctgtttatgcatagataatctctccattcccgtggaacgtttttcctgttcttaagacgtgattttgctgtagaagatggcacttataaccaaagcccaaagtggtatagaaatgctggtttttcagttttcaggagtgggttgatttcagcacctacagtgtacagtcttgtattaagttgttaataaaagtacatgttaaacttaaaaaaaaaaaaaaaaaa

SEQ ID NO: 7 - DNA, 2413 bp, Homo sapiens
  source 1..2413: mol_type = genomic DNA
ttccgtccttccgtccgcggccctgtcagctggagcgcggcgcaggctctgccccggcccggcggctctggccggccgtccagtccgtgcggcggaccccgaggagcctcgatgtggatggccccgcgaagttaagttctgggctcgcgcttccactccgccgcgccttcctcccagtttccgtccgctcgccgcaccggcttcgttcccccaaatctcggaccgtcccttcgcgccccctccccgtccgcccccagtgctgcgttctccccctcttggctctcctgcggctgggggaggggcgggggtcaccatggccgaggcgcctcaggtggtggagatcgacccggacttcgagccgctgccccggccgcgctcgtgcacctggccgctgcccaggccggagtttagccagtccaactcggccacctccagcccggcgccgtcgggcagcgcggctgccaaccccgacgccgcggcgggcctgccctcggcctcggctgccgctgtcagcgccgacttcatgagcaacctgagcttgctggaggagagcgaggacttcccgcaggcgcccggctccgtggcggcggcggtggcggcggcggccgccgcggccgccaccggggggctgtgcggggacttccagggcccggaggcgggctgcctgcacccagcgccaccgcagcccccgccgcccgggccgctgtcgcagcacccgccggtgccccccgccgccgctgggccgctcgcggggcagccgcgcaagagcagctcgtcccgccgcaacgcgtggggcaacctgtcctacgccgacctcatcaccaaggccatcgagagctcggcggagaagcggctcacgctgtcgcagatctacgagtggatggtcaagagcgtgccctacttcaaggataagggtgacagcaacagctcggcgggctggaagaattcaattcgtcataatctgtccctacacagcaagttcattcgtgtgcagaatgaaggaactggaaaaagttcttggtggatgctcaatccagagggtggcaagagcgggaaatctcctaggagaagagctgcatccatggacaacaacagtaaatttgctaagagccgaagccgagctgccaagaagaaagcatctctccagtctggccaggagggtgctggggacagccctggatcacagttttccaaatggcctgcaagccctggctctcacagcaatgatgactttgataactggagtacatttcgccctcgaactagctcaaatgctagtactattagtgggagactctcacccattatgaccgaacaggatgatcttggagaaggggatgtgcattctatggtgtacccgccatctgccgcaaagatggcctctactttacccagtctgtctgagataagcaatcccgaaaacatggaaaatcttttggataatctcaaccttctctcatcaccaacatcattaactgtttcgacccagtcctcacctggcaccatgatgcagcagacgccgtgctactcgtttgcgccaccaaacaccagtttgaattcacccagcccaaactaccaaaaatatacatatggccaatccagcatgagccctttgccccagatgcctatacaaacacttcaggacaataagtcgagttatggaggtatgagtcagtataactgtgcgcctggactcttgaaggagttgctgacttctgactctcctccccataatgacattatgacaccagttgatcctggggtagcccagcccaacagccgggttctgggccagaacgtcatgatgggccctaattcggtcatgtcaacctatggcagccaggcatctcataacaaaatgatgaatcccagctcccatacccaccctggacatgctcagcagacatctgcagttaacgggcgtcccctgccccacacggtaagcaccatgccccacacctcgggtatgaaccgcctgacccaagtgaagacacctgtacaagtgcctctgccccaccccatgcagatgagtgccctggggggctactcctccgtgagcagctgcaatggctatggcagaatgggccttctccaccaggagaagctcccaagtgacttggatggcatgttcattgagcgcttagactgtgacatggaatccatcattcggaatgacctcatggatggagatacattggattttaactttgacaatgtgttgcccaaccaaagcttcccacacagtgtcaagacaacgacacatagctgggtgtcaggctgagggttagtgagcaggttacacttaaaagtacttcagattgtctgacagcaggaactgagagaagcagtccaaagatgtctttcaccaactcccttttagttttctcggttaaaaaaaaaaaaaaaaaaaaaa

SEQ ID NO: 8 - DNA, 3286 bp, Homo sapiens
  source 1..3286: mol_type = genomic DNA
gcgtgtcgggcgcggaagggggaggcggcccggggcgcccgcgagtgaggcgcggggcggcgaagggagcgcgggtggcggcacttgctgccgcggccttggatgggctgggcccccctcgccgctccgcctcctccacacgcgcggcggccgcggcgagggggacgcgccgcccggggcccggcaccttcgggaaccccccggcccggagcctgcggcctgcgccgcctcggccgccgggagccccgtggagcccccgccgccgcgccgccccgcggaccggacgctgagggcactcggggcggggcgcgcgctcgggcagacgtttgcggggaggggggcgcctgccgggccccggcgaccaccttgggggtcgcgggccggctcggggggcgcccagtgcgggccctcgcgggcgccgggcagcgaccagccctgagcggagctgttggccgcggcgggaggcctcccggacgcccccagccccccgaacgctcgcccgggccggcgggagtcggcgccccccgggaggtccgctcggtcgtccgcggcggagcgtttgctcctgggacaggcggtgggaccggggcgtcgccggagacgcccccagcgaagttgggctctccaggtgtgggggtcccggggggtagcgacgtcgcggacccggcctgtgggatgggcggcccggagaagactgcgctcggccgtgttcatacttgtccgtgggcctgaggtccccggaggatgacctagcactgaaaagccccggccggcctccccagggtccccgaggacgaagttgaccctgaccgggccgtctcccagttctgaggcccgggtcccactggaactcgcgtctgagccgccgtcccggacccccggtgcccgccggtccgcagaccctgcaccgggcttggactcgcagccgggactgacgtgtagaacaatcgtttctgttggaagaagggtttttcccttccttttggggtttttgttgccttttttttttcttttttctttgtaaaattttggagaagggaagtcggaacacaaggaaggaccgctcacccgcggactcagggctggcggcgggactccaggaccctgggtccagcatggaggtggtggacccgcagcagctgggcatgttcacggagggcgagctgatgtcggtgggtatggacacgttcatccaccgcatcgactccaccgaggtcatctaccagccgcgccgcaagcgggccaagctcatcggcaagtacctgatgggggacctgctgggggaaggctcttacggcaaggtgaaggaggtgctggactcggagacgctgtgcaggagggccgtcaagatcctcaagaagaagaagttgcgaaggatccccaacggggaggccaacgtgaagaaggaaattcaactactgaggaggttacggcacaaaaatgtcatccagctggtggatgtgttatacaacgaagagaagcagaaaatgtatatggtgatggagtactgcgtgtgtggcatgcaggaaatgctggacagcgtgccggagaagcgtttcccagtgtgccaggcccacgggtacttctgtcagctgattgacggcctggagtacctgcatagccagggcattgtgcacaaggacatcaagccggggaacctgctgctcaccaccggtggcaccctcaaaatctccgacctgggcgtggccgaggcactgcacccgttcgcggcggacgacacctgccggaccagccagggctccccggctttccagccgcccgagattgccaacggcctggacaccttctccggcttcaaggtggacatctggtcggctggggtcaccctctacaacatcaccacgggtctgtaccccttcgaaggggacaacatctacaagttgtttgagaacatcgggaaggggagctacgccatcccgggcgactgtggccccccgctctctgacctgctgaaagggatgcttgagtacgaaccggccaagaggttctccatccggcagatccggcagcacagctggttccggaagaaacatcctccggctgaagcaccagtgcccatcccaccgagcccagacaccaaggaccggtggcgcagcatgactgtggtgccgtacttggaggacctgcacggcgcggacgaggacgaggacctcttcgacatcgaggatgacatcatctacactcaggacttcacggtgcccggacaggtcccagaagaggaggccagtcacaatggacagcgccggggcctccccaaggccgtgtgtatgaacggcacagaggcggcgcagctgagcaccaaatccagggcggagggccgggcccccaaccctgcccgcaaggcctgctccgccagcagcaagatccgccggctgtcggcctgcaagcagcagtgaggctggccgcctgcagcccgtgtccaggagccccgccaggtgcccgcgccaggccctcagtcttcctgccggttccgcccgccctcccggagaggtggccgccatgcttctgtgccgaccacgccccaggacctccggagcgccctgcagggccgggcagggggacagcagggaccgggcgcagccctcccccctcggccgcccggcagtgcacgcggcttgttgacttcgcagccccgggcggagccttcccgggcgggcgtgggaggagggaggcggcctccatgcactttatgtggagactactggccccgcccgtggcctcgtgctccgcagggcgcccagcgccgtccggcggccccgccgcagaccagctggcgggtgtggagaccaggctcctgaccccgccatgcatgcagcgccacctggaagccgcgcggccgctttggttttttgtttggttggttccattttctttttttctttttttttttaagaaaaaataaaaggtggatttgagctgtggctgtgaggggtgtttgggagctgctgggtggcaggggggctgtggggtcgggctcacgtcgcggccgcctttgcgctctcgggtcaccctgctttggcggcccggccggagggcaggaccctcacctctcccccaaggccactgcgctcttgggaccccagagaaaacccggagcaagcaggagtgtgcggtcaatatttatatcatccagaaaagaaaaacacgagaaacgccatcgcgggatggtgcagacgcggcggggactcggagggtgccgtgcgggcgaggccgcccaaatttggcaataaataaagcttgggaagcttggacctgaaaaaaaaaa

SEQ ID NO: 9 - DNA, 6767 bp, Homo sapiens
  source 1..6767: mol_type = genomic DNA
aagtttccaagtggtcaacttgaccgatgctttggcaattgaaaaagggcagaaaggcgcgggctagtgggtggatggggacaaagatctaagtcaccttcttccagcgtgtgagcctgggaggagggtgggggtcctgaggagcaagaggtacgaggaaggaaaaggagagggcttctgggttagtttccacctcctgctttccaactcacggcgctttccttccggaaaggacgctggattcagggcgcgccagtacgcgcagtagcggcccgcgagtcggcaggtgggtagccccggcgcgggaggaaggggaagttaccttcccctcggaagagggcgctggctcccccatcctgcctttataataaggccaccggaggagaggaagcagccagctgccgtctgcgctttgcaaagcatgcagttaggggagcagctcttggtgagctcagtgaacctgcctggcgcgcacttctacccgctggagagtgcgcgaggcggcagcggcgggagcgctggccacctccccagcgcggccccctctcctcagaagttggacttagacaaagcgtccaagaagttttccggcagtctctcctgcgaggcggtgagcggggagcccgcagccgccagcgcaggggcccccgcggccatgcttagtgacaccgacgccggggacgcatttgccagcgctgcggcagtggccaagccggggcccccggacggccgcaagggctccccctgcggggaggaggagctgccctccgccgctgcagccgccgccgccgccgccgccgcggctgcggccactgcgcgctactccatggacagcctgagctccgagcggtactacctccagtcccccggtcctcaggggtcggagctggctgcgccctgctcactcttcccgtaccaggcggcggctggggcgccccacggacctgtgtacccggctcctaacggggcgcgctacccctacggctccatgctgccccccggcggcttccccgcggctgtgtgcccacccgggagggcgcagttcggcccaggagccggtgcgggcagtggcgcgggcggtagcagcggcgggggcggcggcccgggcacctatcagtacagccagggggctccgctctacgggccgtaccctggagccgcagcggcgggatcttgcggaggactggggggcctgggggttccaggttctggcttccgtgcccacgtctacctgtgcaaccggcctctgtggctcaaattccaccgccaccaaactgagatgatcattacgaaacagggcaggtgagcgcagcgtggaggggcccctgggttcggggataaagggtgacgtgtggtcctggggaaggtccgggatgagggagctgaacccagttgttccgcgcggtgcttagagtgtttcaccgcgcgcaataaatctccgtagacaccgcatctccaatgcggtgtccctctgtgtcagtgccccggcggctcttgcagggtgccaatgttacggctgtacaccgcttttccctcccatcatcctcacctgaacagacctggaggaggcggaaatggaaattagggcatgtccacaagctggattcgttagatcctcctgctcggcggtatgcttgtgcatgcctgcatgccggcaaggagccacggatagggaaggctcaagagctggccacctgagcgcagtagatgggctcccgcagttttaggcgccagggtctccacggggcgtctccgggaggtgggcatgaaggctagagcgccggcctcggaagctcggtcggagtaggtggttagatctgccctggagccagacctggctcgggttcggtgcgcgagaaagttctgatatacatccaactgctaacactggctacttctggggaaagggaggggtgggtgctgagagaggggcactcaaaggggacttttagcctaaagttttaatatatatttttaacaagaataacctaatattgttctctggtacttttcaaaatggtgcatttaaaaattagtagtttttaacattctaggagaaaaattttaagagcgtctgaaagggccgagaatatgagccttcggaagcacgcgcgaatttggaatataccgatgttggggcaagcttttttttttttttttttttttttttttttttttttttttgaaaagacggaaaggttccaagagttgccaactcaaaaatattttacatagtttcagaccacttgatctaccagcattctgttcactgcaaacttttaaatgtgttccgaccctatcccaggtgtctggggaacccgctggggcctgggcctgttctaggacatcccaattaaaatcgatttttctgattctattcccttgcacaggcgcatgtttcctttcttgagcttcaacataaacggactcaatcccactgcccactacaatgtgttcgtagaggtggtgctggcggaccccaaccactggcgcttccaggggggcaaatgggtgacctgtggcaaagccgacaataacatgcagggtgagcagagaagaggctcgggccggggaggaacgggcgggaagaaatcgtaaccctcgactcacacaactcacatttaaatgtagcactttttttttccccttccattctgaggcctagaggtgttagtatgagtgtctttgagttgcttgtttgacggagaggagagtttgctaagtcagatttcttgtctgccaatatgtagatatttagaacctttaactaagacatcaccccaccccccaatccctacgtttaacaaatcagtagtcataagctctccaggtgggaagggctcctgggattctaatgttcacttgagaaagcccagccaaagtttagttcacccataaatatccaactgtcttccatcggatgttgcccttacagctttagaaggccccaaattgaccttcaagagtcatctcttgttagctccgtttctaaattctgaaatgccattcaggggagtccctagtgcaaggaaggttggaagcacaggggcctgggagggatatggatgtagtcctgctggtctccactggcctctttaagcaacttttactgggagaccaactgtaagtctagctcttatatcttgctcatagctaagagacatccctccgctttctccatttgtaaacagccctatatgcttgggttttgtgttttgtttcattttctcttaggcaacaaaatgtatgttcacccagagtctcctaatactggttcccactggatgagacaggagatttcattcgggaaattaaaactcaccaataacaaaggcgcaaataacaacaacacccaggtagagtgacagagcaggaggggatatcttctggctttgactataaggcttttttctaataagagtccctactcttttcactgtatttataatatttgcatttgtgacctgtttgctcgcctatttctaaccatttttgttcttttgacctttctcatcttcactttcttattggatttcgataacagtgagttgactattaagaacagaaatagcgaagtattttgggaatttaggaaaccaagaggaaagcatatctatcacaaccacatacccagctatgatttaaatttcaaaaaaaaagtgggggggcaataatgagacctttaaacttgcaataaacaaagctgttagtgaggagcatttagaagtccaataccaaaatacataatttgtcaaaatctaattttgttgaaccactaagaggctttttagatttagcaatttttttctgtactctttccagatgatagtcttacaatccttacacaaataccaaccccgactgcatattgttgaagttacagaggatggcgtggaggacttgaatgagccctcaaagacccagacttttaccttctcagaaacgcaattcattgcagtgactgcctaccaaaacaccgatgtgagtgtcccagacatctcaagaatctctaaagctaaggtccagcatgataaatcactcaatgactgtttttctcccctatctagattactcaactaaagattgatcataacccctttgcaaaaggcttcagagacaactatgattcgtaagtgcagcttttatccacacttgcctgatcatctctgagcaggacatacatcaacaggcactttgctgataatgtattttaggaagagcttttacctttgggatttttacatatttttctttttccaaaattttttcctttactaatcttgctttagatttttctcagaaaggttgtgttaatttctgaagaaatgttaaggacttaaaaatgaagaggtttttttagcatttgagtgaagatttgaaattttaagaatctgcatttatatatacctttcttttcatttgatccatttttttatcctcccaagagcagatattattactctcccccacccccacttttttttttaacataagaaaaaactgaaactaagaggatgtaatttcacaacacgaaatagcaaggccctgctctttttaaaatctgagttttctaccgccacagccagtgttttttccatcacattgacaaaggaggtttgatctgagtttttcgtgttctaggactagtaaaggtagattttctatagtttaaatacttgatgcctaggaggaaactttttcttgcatggtgggaaatttttcccaataagccaagagtccagctaaaatgggccagtgcatctcctgcctctgttctttcagcccaacagaccagcactttcggtgtagataaccaacacaagcctttttcatttctgggaggtggtttgtttggggacaacattagggtttttttttttttttaagtgtttctctttatattgtagcatgtacaccgcttcagaaaatgacaggttaactccatctcccacggattctcctagatcccatcagattgtccctggaggtcggtacggcgttcaatccttcttcccggagccctttgtcaacactttacctcaagcccgctattataatggcgagagaaccgtgccacagaccaacggcctcctttcaccccaacagagcgaagaggtggccaaccctccccagcggtggcttgtcacgcctgtccagcaacctgggaccaacaaactagacatcagttcctatgaatctgaatatacttctagcacattgctcccatatggcattaaatccttgccccttcagacatcccatgccctggggtattacccagacccaacctttcctgcaatggcagggtggggaggtcgaggttcttaccagaggaagatggcagctggactaccatggacctccagaacaagccccactgtgttctctgaagatcagctctccaaggagaaagtgaaagaggaaattggctcttcttggatagagacacccccttccatcaaatctctagattccaatgattcaggagtatacaccagtgcttgtaagcgaaggcggctgtctcctagcaactccagtaatgaaaattcaccctccataaagtgtgaggacattaatgctgaagagtatagtaaagacacctcaaaaggcatgggagggtattatgctttttacacaactccctaaagagttattttaacctcaaaaattagctaactttttgcagatggacttggtggtgttttttgttgtcttctttgcctaggttgccaaaaagatgtttgccttccaccttgatgcatcctgttttgtgcaattctctaaaagaaggtgccaaagctttttgattgctgcaggtaactgaaacaaacctagcatttttaaaaaataagattaatggaagactttaaggtattttaaaattcgaagggtatccaaggttctgtatttatttattggggagacactaacccttcaaagaagcaggctgtgaacattgggtgcccagtgctatcagatgagttaaaacctttgattctcatttctatttgtaaattcttaagcaaatagaagccgagtgttaaggtgttttgcttctgaaagagggctgtgccttccgtttcagaaggagacattttgctgttacattctgccaggggcaaaagatactaggcccaggagtcaagaaaagcttttgtgaaagtgatagtttcacctgactttgattccttaacccccggcttttggaacaagccatgtttgccctagtccaggattgcctcacttgagacttgctaggcctctgctgtgtgctggggtggccagtgggactcaggagagagcaagctaaggagtcaccaaaaaaaaaaaaaaaaaaaagggagaatttaaaagtgtacagttgtgtgtttagatacactatagaataatgtggtatatattgtacaaatagtctacataggtgtctgggataatgtaaaactggtgctttggctttgtaaagaatttgcaaatcacttaacagctgcaggggcaaggggagagtttcatcatccccatgatatttgggaatattctgtttacttcttagatagttaagaatgtattcagctactatgtactaacttgaaccgtgtttaaggaaaactcctatttcatcctcttcttgcgccatcccctctccctaacttggtaatgtgaagaaactaaaacctgataccacagctcctataggcattttagagatcttggatttttatgtacagtcttagtcatttttaataaatgtggttcagtaagggaacgga

SEQ ID NO: 10 - DNA, 2471 bp, Homo sapiens
  source 1..2471: mol_type = genomic DNA
ggggacgaagggaagctccagcgtgtggccccggcgagtgcggataaaagccgccccgccgggctcgggcttcattctgagccgagcccggtgccaagcgcagctagctcagcaggcggcagcggcggcctgagcttcagggcagccagctccctcccggtctcgccttccctcgcggtcagcatgaaagccttcagtcccgtgaggtccgttaggaaaaacagcctgtcggaccacagcctgggcatctcccggagcaaaacccctgtggacgacccgatgagcctgctatacaacatgaacgactgctactccaagctcaaggagctggtgcccagcatcccccagaacaagaaggtgagcaagatggaaatcctgcagcacgtcatcgactacatcttggacctgcagatcgccctggactcgcatcccactattgtcagcctgcatcaccagagacccgggcagaaccaggcgtccaggacgccgctgaccaccctcaacacggatatcagcatcctgtccttgcaggtaagacctgctccggggtccccgccccgccgccgcacactcccgcggtcgtctgggctgtcactaggagatccgtagcccagacggtgactttcgtatgagctatttaactttattttcttcagaatctgctgtagattgagctgtgcgtgaaattgctagtaagttctgacatgttaatgcgtctgtctttaaatctgaattgttaccataaacgtgtttaatggaacttgctggtctgtggactacaaaaaaaaaaaaaaaaaaaaaaaaaccctttctacttaacattgtcttaacctcgtactctttatcctctttctttccaggcttctgaattcccttctgagttaatgtcaaatgacagcaaagcactgtgtggctgaataagcggtgagtgtttgcttgtgccacccgtgggtaaactgcccctcggtgtgtgtgcgcgcgcgcgcatgtgtttttgcttgtgtatctataaaatgtctgatttggtaaatgcatgcttacttcgcggtgttacccgtactacattgtctcactagacatgaaggagcttgtagctttgggtgctcgagatcacagaacattttcctttaaaaggaaatgatgccaataacttactacgaaggcggccgaggaacgtgtgtattggctttgtagcaaatgtaatgccctggatcttcctacgagtcctctggtactatgaggtactaacctccactgtaattaatcttaccgccacaaattccatagtgatcctccttccctaaaactatagtcctctgggattctctgggctagttgaggattgctaccctgtgccttcaaccctgtgatgtgggatcccagacttccctatctgttaactaaagggctgttttcaatcaaataattgttacgagaagcagactggcgcctgtagcactgctgttggagatccaaataggagattgggttgggaagtttttcccttgagtctctgctattttaatgtttaatttgcgctgtcgaggcgagtgtgtgtgttgcatctggacgccagggtttgcccaatctttgagtgtttggttaaatgttcaaactgtggcttcctcccggcgccagtcgcccgcctctgcccttaggttacattctcttaaacatgcctttctcccccactctttcgcaggtgttcatgatttcttttattctttgcacaacaacaacaacaacaaattcacggaatcttttaagtgctgaacttatttttcaaccatttcacaaggaggacaagttgaatggacctttttaaaaagaaaaaaaaaatggaaggaaaactaagaatgatcatcttcccagggtgttctcttacttggactgtgatattcgttatttatgaaaaagacttttaaatgccctttctgcagttggaaggttttctttatatactattcccaccatggggagcgaaaacgttaaaatcacaaggaattgcccaatctaagcagactttgccttttttcaaaggtggagcgtgaataccagaaggatccagtattcagtcacttaaatgaagtcttttggtcagaaattacctttttgacacaagcctactgaatgctgtgtatatatttatatataaatatatctatttgagtgaaaccttgtgaactctttaattagagttttcttgtatagtggcagagatgtctatttctgcattcaaaagtgtaatgatgtacttattcatgctaaactttttataaaagtttagttgtaaacttaacccttttatacaaaataaatcaagtgtgtttattgaatggtgattgcctgctttatttcagaggaccagtgctttgatttttattatgctatgttataactgaacccaaataaatacaagttcaaatttatgtagactgtataagattataataaaacatgtctgaagtcaa

SEQ ID NO: 11 - DNA, 4018 bp, Homo sapiens
  source 1..4018: mol_type = genomic DNA
caggcagcgctgcgtcctgctgcgcacgtgggaagccctggccccggccacccccgcgatgccgcgcgctccccgctgccgagccgtgcgctccctgctgcgcagccactaccgcgaggtgctgccgctggccacgttcgtgcggcgcctggggccccagggctggcggctggtgcagcgcggggacccggcggctttccgcgcgctggtggcccagtgcctggtgtgcgtgccctgggacgcacggccgccccccgccgccccctccttccgccaggtgtcctgcctgaaggagctggtggcccgagtgctgcagaggctgtgcgagcgcggcgcgaagaacgtgctggccttcggcttcgcgctgctggacggggcccgcgggggcccccccgaggccttcaccaccagcgtgcgcagctacctgcccaacacggtgaccgacgcactgcgggggagcggggcgtgggggctgctgctgcgccgcgtgggcgacgacgtgctggttcacctgctggcacgctgcgcgctctttgtgctggtggctcccagctgcgcctaccaggtgtgcgggccgccgctgtaccagctcggcgctgccactcaggcccggcccccgccacacgctagtggaccccgaaggcgtctgggatgcgaacgggcctggaaccatagcgtcagggaggccggggtccccctgggcctgccagccccgggtgcgaggaggcgcgggggcagtgccagccgaagtctgccgttgcccaagaggcccaggcgtggcgctgcccctgagccggagcggacgcccgttgggcaggggtcctgggcccacccgggcaggacgcgtggaccgagtgaccgtggtttctgtgtggtgtcacctgccagacccgccgaagaagccacctctttggagggtgcgctctctggcacgcgccactcccacccatccgtgggccgccagcaccacgcgggccccccatccacatcgcggccaccacgtccctgggacacgccttgtcccccggtgtacgccgagaccaagcacttcctctactcctcaggcgacaaggagcagctgcggccctccttcctactcagctctctgaggcccagcctgactggcgctcggaggctcgtggagaccatctttctgggttccaggccctggatgccagggactccccgcaggttgccccgcctgccccagcgctactggcaaatgcggcccctgtttctggagctgcttgggaaccacgcgcagtgcccctacggggtgctcctcaagacgcactgcccgctgcgagctgcggtcaccccagcagccggtgtctgtgcccgggagaagccccagggctctgtggcggcccccgaggaggaggacacagacccccgtcgcctggtgcagctgctccgccagcacagcagcccctggcaggtgtacggcttcgtgcgggcctgcctgcgccggctggtgcccccaggcctctggggctccaggcacaacgaacgccgcttcctcaggaacaccaagaagttcatctccctggggaagcatgccaagctctcgctgcaggagctgacgtggaagatgagcgtgcgggactgcgcttggctgcgcaggagcccaggggttggctgtgttccggccgcagagcaccgtctgcgtgaggagatcctggccaagttcctgcactggctgatgagtgtgtacgtcgtcgagctgctcaggtctttcttttatgtcacggagaccacgtttcaaaagaacaggctctttttctaccggaagagtgtctggagcaagttgcaaagcattggaatcagacagcacttgaagagggtgcagctgcgggagctgtcggaagcagaggtcaggcagcatcgggaagccaggcccgccctgctgacgtccagactccgcttcatccccaagcctgacgggctgcggccgattgtgaacatggactacgtcgtgggagccagaacgttccgcagagaaaagagggccgagcgtctcacctcgagggtgaaggcactgttcagcgtgctcaactacgagcgggcgcggcgccccggcctcctgggcgcctctgtgctgggcctggacgatatccacagggcctggcgcaccttcgtgctgcgtgtgcgggcccaggacccgccgcctgagctgtactttgtcaaggtggatgtgacgggcgcgtacgacaccatcccccaggacaggctcacggaggtcatcgccagcatcatcaaaccccagaacacgtactgcgtgcgtcggtatgccgtggtccagaaggccgcccatgggcacgtccgcaaggccttcaagagccacgtctctaccttgacagacctccagccgtacatgcgacagttcgtggctcacctgcaggagaccagcccgctgagggatgccgtcgtcatcgagcagagctcctccctgaatgaggccagcagtggcctcttcgacgtcttcctacgcttcatgtgccaccacgccgtgcgcatcaggggcaagtcctacgtccagtgccaggggatcccgcagggctccatcctctccacgctgctctgcagcctgtgctacggcgacatggagaacaagctgtttgcggggattcggcgggacgggctgctcctgcgtttggtggatgatttcttgttggtgacacctcacctcacccacgcgaaaaccttcctcaggaccctggtccgaggtgtccctgagtatggctgcgtggtgaacttgcggaagacagtggtgaacttccctgtagaagacgaggccctgggtggcacggcttttgttcagatgccggcccacggcctattcccctggtgcggcctgctgctggatacccggaccctggaggtgcagagcgactactccagctatgcccggacctccatcagagccagtctcaccttcaaccgcggcttcaaggctgggaggaacatgcgtcgcaaactctttggggtcttgcggctgaagtgtcacagcctgtttctggatttgcaggtgaacagcctccagacggtgtgcaccaacatctacaagatcctcctgctgcaggcgtacaggtttcacgcatgtgtgctgcagctcccatttcatcagcaagtttggaagaaccccacatttttcctgcgcgtcatctctgacacggcctccctctgctactccatcctgaaagccaagaacgcagggatgtcgctgggggccaagggcgccgccggccctctgccctccgaggccgtgcagtggctgtgccaccaagcattcctgctcaagctgactcgacaccgtgtcacctacgtgccactcctggggtcactcaggacagcccagacgcagctgagtcggaagctcccggggacgacgctgactgccctggaggccgcagccaacccggcactgccctcagacttcaagaccatcctggactgatggccacccgcccacagccaggccgagagcagacaccagcagccctgtcacgccgggctctacgtcccagggagggaggggcggcccacacccaggcccgcaccgctgggagtctgaggcctgagtgagtgtttggccgaggcctgcatgtccggctgaaggctgagtgtccggctgaggcctgagcgagtgtccagccaagggctgagtgtccagcacacctgccgtcttcacttccccacaggctggcgctcggctccaccccagggccagcttttcctcaccaggagcccggcttccactccccacataggaatagtccatccccagattcgccattgttcacccctcgccctgccctcctttgccttccacccccaccatccaggtggagaccctgagaaggaccctgggagctctgggaatttggagtgaccaaaggtgtgccctgtacacaggcgaggaccctgcacctggatgggggtccctgtgggtcaaattggggggaggtgctgtgggagtaaaatactgaatatatgagtttttcagttttgaaaaaaa

SEQ ID NO: 12 - DNA, 2335 bp, Homo sapiens
  source 1..2335: mol_type = genomic DNA
gttattctctggaacatgaaacattctgttgtgctcatatcatgcaaattatcactagtaggagagcagagagtggaaatgttccaggtataaagacccacaagataaagaagctcagagtcgttagaaacaggagcagatgtacagggtttgcctgactcacactcaaggttgcataagcaagatttcaaaattaatcctattctggagacctcaacccaatgtacaatgttcctgactggaaaagaagaactatatttttctgattttttttttcaaatctttaccattagttgccctgtatctccgccttcactttctgcaggaaactttatttcctacttctgcatgccaagtttctacctctagatctgtttggttcagttgctgagaagcctgacataccaggactgcctgagacaagccacaagctgaacagagaaagtggattgaacaaggacgcatttccccagtacatccacaacatgctgtccacatctcgttctcggtttatcagaaataccaacgagagcggtgaagaagtcaccaccttttttgattatgattacggtgctccctgtcataaatttgacgtgaagcaaattggggcccaactcctgcctccgctctactcgctggtgttcatctttggttttgtgggcaacatgctggtcgtcctcatcttaataaactgcaaaaagctgaagtgcttgactgacatttacctgctcaacctggccatctctgatctgctttttcttattactctcccattgtgggctcactctgctgcaaatgagtgggtctttgggaatgcaatgtgcaaattattcacagggctgtatcacatcggttattttggcggaatcttcttcatcatcctcctgacaatcgatagatacctggctattgtccatgctgtgtttgctttaaaagccaggacggtcacctttggggtggtgacaagtgtgatcacctggttggtggctgtgtttgcttctgtcccaggaatcatctttactaaatgccagaaagaagattctgtttatgtctgtggcccttattttccacgaggatggaataatttccacacaataatgaggaacattttggggctggtcctgccgctgctcatcatggtcatctgctactcgggaatcctgaaaaccctgcttcggtgtcgaaacgagaagaagaggcatagggcagtgagagtcatcttcaccatcatgattgtttactttctcttctggactccctataatattgtcattctcctgaacaccttccaggaattcttcggcctgagtaactgtgaaagcaccagtcaactggaccaagccacgcaggtgacagagactcttgggatgactcactgctgcatcaatcccatcatctatgccttcgttggggagaagttcagaaggtatctctcggtgttcttccgaaagcacatcaccaagcgcttctgcaaacaatgtccagttttctacagggagacagtggatggagtgacttcaacaaacacgccttccactggggagcaggaagtctcggctggtttataaaacgaggagcagtttgattgttgtttataaagggagataacaatctgtatataacaacaaacttcaagggtttgttgaacaatagaaacctgtaaagcaggtgcccaggaacctcagggctgtgtgtactaatacagactatgtcacccaatgcatatccaacatgtgctcagggaataatccagaaaaactgtgggtagagactttgactctccagaaagctcatctcagctcctgaaaaatgcctcattaccttgtgctaatcctctttttctagtcttcataatttcttcactcaatctctgattctgtcaatgtcttgaaatcaagggccagctggaggtgaagaagagaatgtgacaggcacagatgaatgggagtgagggatagtggggtcagggctgagaggagaaggagggagacatgagcatggctgagcctggacaaagacaaaggtgagcaaagggctcacgcattcagccaggagatgatactggtccttagccccatctgccacgtgtatttaaccttgaagggttcaccaggtcagggagagtttgggaactgcaataacctgggagttttggtggagtccgatgattctcttttgcataagtgcatgacatatttttgctttattacagtttatctatggcacccatgcaccttacatttgaaatctatgaaatatcatgctccattgttcagatgcttcttaggccacatccccctgtctaaaaattcagaaaatttttgtttataaaaga

SEQ ID NO: 13 - DNA, 1657 bp, Homo sapiens
  source 1..1657: mol_type = genomic DNA
tctcacaggaagccacgcacccttgaaaggcaccgggtccttcttagcatcgtgcttcctgagcaagcctggcattgcctcacagaccttcctcagagccgctttcagaaaagcaagctgcttctggttgggcccagacctgccttgaggagcctgtagagttaaaaaatgaaccccacggatatagcagacaccaccctcgatgaaagcatatacagcaattactatctgtatgaaagtatccccaagccttgcaccaaagaaggcatcaaggcatttggggagctcttcctgcccccactgtattccttggtttttgtatttggtctgcttggaaattctgtggtggttctggtcctgttcaaatacaagcggctcaggtccatgactgatgtgtacctgctcaaccttgccatctcggatctgctcttcgtgttttccctccctttttggggctactatgcagcagaccagtgggtttttgggctaggtctgtgcaagatgatttcctggatgtacttggtgggcttttacagtggcatattctttgtcatgctcatgagcattgatagatacctggcaattgtgcacgcggtgttttccttgagggcaaggaccttgacttatggggtcatcaccagtttggctacatggtcagtggctgtgttcgcctcccttcctggctttctgttcagcacttgttatactgagcgcaaccatacctactgcaaaaccaagtactctctcaactccacgacgtggaaggttctcagctccctggaaatcaacattctcggattggtgatccccttagggatcatgctgttttgctactccatgatcatcaggaccttgcagcattgtaaaaatgagaagaagaacaaggcggtgaagatgatctttgccgtggtggtcctcttccttgggttctggacaccttacaacatagtgctcttcctagagaccctggtggagctagaagtccttcaggactgcacctttgaaagatacttggactatgccatccaggccacagaaactctggcttttgttcactgctgccttaatcccatcatctacttttttctgggggagaaatttcgcaagtacatcctacagctcttcaaaacctgcaggggcctttttgtgctctgccaatactgtgggctcctccaaatttactctgctgacacccccagctcatcttacacgcagtccaccatggatcatgatctccatgatgctctgtagaaaaatgaaatggtgaaatgcagagtcaatgaactttccacattcagagcttacttaaaattgtattttagtaagagattcctgagccagtgtcaggaggaaggcttacacccacagtggaaagacagcttctcatcctgcaggcagctttttctctcccactagacaagtccagcctggcaagggttcacctgggctgaggcatccttcctcacaccaggcttgcctgcaggcatgagtcagtctgatgagaactctgagcagtgcttgaatgaagttgtaggtaatattgcaaggcaaagactattcccttctaacctgaactgatgggtttctccagagggaattgcagagtactggctgatggagtaaatcgctaccttttgctgtggcaaatgggccctct

SEQ ID NO: 14 - protein, 750 aa, Homo sapiens
MWNLLHETDSAVATARRPRWLCAGALVLAGGFFLLGFLFGWFIKSSNEATNITPKHNMKAFLDELKAENIKKFLYNFTQIPHLAGTEQNFQLAKQIQSQWKEFGLDSVELAHYDVLLSYPNKTHPNYISIINEDGNEIFNTSLFEPPPPGYENVSDIVPPFSAFSPQGMPEGDLVYVNYARTEDFFKLERDMKINCSGKIVIARYGKVFRGNKVKNAQLAGAKGVILYSDPADYFAPGVKSYPDGWNLPGGGVQRGNILNLNGAGDPLTPGYPANEYAYRRGIAEAVGLPSIPVHPIGYYDAQKLLEKMGGSAPPDSSWRGSLKVPYNVGPGFTGNFSTQKVKMHIHSTNEVTRIYNVIGTLRGAVEPDRYVILGGHRDSWVFGGIDPQSGAAVVHEIVRSFGTLKKEGWRPRRTILFASWDAEEFGLLGSTEWAEENSRLLQERGVAYINADSSIEGNYTLRVDCTPLMYSLVHNLTKELKSPDEGFEGKSLYESWTKKSPSPEFSGMPRISKLGSGNDFEVFFQRLGIASGRARYTKNWETNKFSGYPLYHSVYETYELVEKFYDPMFKYHLTVAQVRGGMVFELANSIVLPFDCRDYAVVLRKYADKIYSISMKHPQEMKTYSVSFDSLFSAVKNFTEIASKFSERLQDFDKSNPIVLRMMNDQLMFLERAFIDPLGLPDRPFYRHVIYAPSSHNKYAGESFPGIYDALFDIESKVDPSKAWGEVKRQIYVAAFTVQAAAETLSEVA

SEQ ID NO: 15 - protein, 123 aa, Homo sapiens
MKAVLLALLMAGLALQPGTALLCYSCKAQVSNEDCLQVENCTQLGEQCWTARIRAVGLLTVISKGCSLNCVDDSQDYYVGKKNITCCDTDLCNASGAHALQPAAAILALLPALGLLLWGPGQL

SEQ ID NO: 16 - protein, 622 aa, Homo sapiens [sequence omitted]

SEQ ID NO: 17 - protein, 556 aa, Homo sapiens [sequence omitted]

SEQ ID NO: 18 - protein, 297 aa, Homo sapiens
MTTPRNSVNGTFPAEPMKGPIAMQSGPKPLFRRMSSLVGPTQSFFMRESKTLGAVQIMNGLFHIALGGLLMIPAGIYAPICVTVWYPLWGGIMYIISGSLLAATEKNSRKCLVKGKMIMNSLSLFAAISGMILSIMDILNIKISHFLKMESLNFIRAHTPYINIYNCEPANPSEKNSPSTQYCYSIQSLFLGILSVMLIFAFFQELVIAGIVENEWKRTCSRPKSNIVLLSAEEKKEQTIEIKEEVVGLTETSSQPKNEEDIEIIPIQEEEEEETETNFPEPPQDQESSPIENDSSP

SEQ ID NO: 19 - protein, 937 aa, Homo sapiens
MHRPRRRGTRPPLLALLAALLLAARGAAAQETELSVSAELVPTSSWNISSELNKDSYLTLDEPMNNITTSLGQTAELHCKVSGNPPPTIRWFKNDAPVVQEPRRLSFRSTIYGSRLRIRNLDTTDTGYFQCVATNGKEVVSSTGVLFVKFGPPPTASPGYSDEYEEDGFCQPYRGIACARFIGNRTVYMESLHMQGEIENQITAAFTMIGTSSHLSDKCSQFAIPSLCHYAFPYCDETSSVPKPRDLCRDECEILENVLCQTEYIFARSNPMILMRLKLPNCEDLPQPESPEAANCIRIGIPMADPINKNHKCYNSTGVDYRGTVSVTKSGRQCQPWNSQYPHTHTFTALRFPELNGGHSYCRNPGNQKEAPWCFTLDENFKSDLCDIPACDSKDSKEKNKMEILYILVPSVAIPLAIALLFFFICVCRNNQKSSSAPVQRQPKHVRGQNVEMSMLNAYKPKSKAKELPLSAVRFMEELGECAFGKIYKGHLYLPGMDHAQLVAIKTLKDYNNPQQWTEFQQEASLMAELHHPNIVCLLGAVTQEQPVCMLFEYINQGDLHEFLIMRSPHSDVGCSSDEDGTVKSSLDHGDFLHIAIQIAAGMEYLSSHFFVHKDLAARNILIGEQLHVKISDLGLSREIYSADYYRVQSKSLLPIRWMPPEAIMYGKFSSDSDIWSFGVVLWEIFSFGLQPYYGFSNQEVIEMVRKRQLLPCSEDCPPRMYSLMTECWNEIPSRRPRFKDIHVRLRSWEGLSSHTSSTTPSGGNATTQTTSLSASPVSNLSNPRYPNYMFPSQGITPQGQIAGFIGPPIPQNQRFIPINGYPIPPGYAAFPAAHYQPTGPPRVIQHCPPPKSRSPSSASGSTSTGHVTSLPSSGSNQEANIPLLPHMSIPNHPGGMGITVFGNKSQKPYKIDSKQASLLGDANIHGHTESMISAEL

SEQ ID NO: 20 - protein, 168 aa, Homo sapiens
MGHHHHHHHHHHSSGHIEGRHMRRVPGVAPTLVRSASETSEKRPFMCAYPGCNKRYFKLSHLQMHSRKHTGEKPYQCDFKDCERRFFRSDQLKRHQRRHTGVKPFQCKTCQRKFSRSDHLKTHTRTHTGEKPFSCRWPSCQKKFARSDELVRHHNMHQRNMTKLQLAL

SEQ ID NO: 21 - protein, 347 aa, Homo sapiens
DPNFWLQVQESVTVQEGLCVLVPCTFFHPIPYYDKNSPVHGYWFREGAIISRDSPVATNKLDQEVQEETQGRFRLLGDPSRNNCSLSIVDARRRDNGSYFFRMERGSTKYSYKSPQLSVHVTDLTHRPKILIPGTLEPGHSKNLTCSVSWACEQGTPPIFSWLSAAPTSLGPRTTHSSVLIITPRPQDHGTNLTCQVKFAGAGVTTERTIQLNVTYVPQNPTTGIFPGDGSGKQETRAGVVHGAIGGAGVTALLALCLCLIFFIVKTHRRKAARTAVGRNDTHPTTGSASPKHQKKSKLHGPTETSSCSGAAPTVEMDEELHYASLNFHGMNPSKDTSTEYSEVRTQ

SEQ ID NO: 22 - protein, 11 aa, synthetic construct
  REGION 1..11: note = anti-CD19 scFV CDRL1
RASQDISKYLN

SEQ ID NO: 23 - protein, 7 aa, synthetic construct
  REGION 1..7: note = anti-CD19 scFVCDRL2
SRLHSGV

SEQ ID NO: 24 - protein, 9 aa, synthetic construct
  REGION 1..9: note = anti-CD19 scFVCDRL3
GNTLPYTFG

SEQ ID NO: 25 - protein, 5 aa, synthetic construct
  REGION 1..5: note = anti-CD19 scFVCDRH1
DYGVS

SEQ ID NO: 26 - protein, 16 aa, synthetic construct
  REGION 1..16: note = anti-CD19 scFVCDRH2
VTWGSETTYYNSALKS

SEQ ID NO: 27 - protein, 7 aa, synthetic construct
  REGION 1..7: note = anti-CD19 scFVCDRH3
YAMDYWG

SEQ ID NO: 28 - DNA, 734 bp, synthetic construct
  misc_feature 1..734: note = anti-CD19 scFv (VH-VL) FMC63
  source 1..734: mol_type = other DNA
cacatccagatgacccagaccacctccagcctgagcgccagcctgggcgaccgggtgaccatcagctgccgggccagccaggacatcagcaagtacctgaactggtatcagcagaagcccgacggcaccgtcaagctgctgatctaccacaccagccggctgcacagcggcgtgcccagccggtttagcggcagcggctccggcaccgactacagcctgaccatctccaacctggaacaggaagatatcgccacctacttttgccagcagggcaacacactgccctacacctttggcggcggaacaaagctggaaatcaccggcagcacctccggcagcggcaagcctggcagcggcgagggcagcaccaagggcgaggtgaagctgcaggaaagcggccctggcctggtggcccccagccagagcctgagcgtgacctgcaccgtgagcggcgtgagcctgcccgactacggcgtgagctggatccggcagccccccaggaagggcctggaatggctgggcgtgatctggggcagcgagaccacctactacaacagcgccctgaagagccggctgaccatcatcaaggacaacagcaagagccaggtgttcctgaagatgaacagcctgcagaccgacgacaccgccatctactactgcgccaagcactactactacggcggcagctacgccatggactactggggccagggcaccagcgtgaccgtgagcag

SEQ ID NO: 29 - protein, 245 aa, synthetic construct
  REGION 1..245: note = anti-CD19 scFv (VH-VL) FMC63
DIQMTQTTSSLSASLGDRVTISCRASQDISKYLNWYQQKPDGTVKLLIYHTSRLHSGVPSRFSGSGSGTDYSLTISNLEQEDIATYFCQQGNTLPYTFGGGTKLEITGSTSGSGKPGSGEGSTKGEVKLQESGPGLVAPSQSLSVTCTVSGVSLPDYGVSWIRQPPRKGLEWLGVIWGSETTYYNSALKSRLTIIKDNSKSQVFLKMNSLQTDDTAIYYCAKHYYYGGSYAMDYWGQGTSVTVSS

SEQ ID NO: 30 - protein, 11 aa, synthetic construct
  REGION 1..11: note = anti-ROR1 scFV CDRL1
ASGFDFSAYYM

SEQ ID NO: 31 - protein, 7 aa, synthetic construct
  REGION 1..7: note = anti-ROR1 scFV CDRL2
TIYPSSG

SEQ ID NO: 32 - protein, 9 aa, synthetic construct
  REGION 1..9: note = anti-ROR1 scFV CDRL3
ADRATYFCA

SEQ ID NO: 33 - protein, 6 aa, synthetic construct
  REGION 1..6: note = anti-ROR1 scFV CDRH1
DTIDWY

SEQ ID NO: 34 - protein, 16 aa, synthetic construct
  REGION 1..16: note = anti-ROR1 scFV CDRH2
VQSDGSYTKRPGVPDR

SEQ ID NO: 35 - protein, 8 aa, synthetic construct
  REGION 1..8: note = anti-ROR1 scFV CDRH3
YIGGYVFG

SEQ ID NO: 36 - DNA, 123 bp, Homo sapiens
  source 1..123: mol_type = genomic DNA
cggagcaagcggagcagaggcggccacagcgactacatgaacatgacccccagacggcctggccccacccggaagcactaccagccctacgccccacccagggactttgccgcctacagaagc

SEQ ID NO: 37 - DNA, 1476 bp, synthetic construct
  misc_feature 1..1476: note = P28z CAR
  source 1..1476: mol_type = other DNA
gtggcctcaccgttgacccgctttctgtcgctgaacctgctgctgctgggtgagtcgattatcctggggagtggagaagctgaggtgcagctgcagcagtcaggacctgaactggtgaagcctgggacttcagtgaggatatcctgcaagacttctggatacacattcactgaatataccatacactgggtgaagcagagccatggaaagagccttgagtggattggaaacatcaatcctaacaatggtggtaccacctacaatcagaagttcgaggacaaggccacattgactgtagacaagtcctccagtacagcctacatggagctccgcagcctaacatctgaggattctgcagtctattattgtgcagctggttggaactttgactactggggccaagggaccacggtcaccgtctcctcaggtggaggtggatcaggtggaggtggatctggtggaggtggatctgacattgtgatgacccagtctcacaaattcatgtccacatcagtaggagacagggtcagcatcatctgtaaggccagtcaagatgtgggtactgctgtagactggtatcaacagaaaccaggacaatctcctaaactactgatttattgggcatccactcggcacactggagtccctgatcgcttcacaggcagtggatctgggacagacttcactctcaccattactaatgttcagtctgaagacttggcagattatttctgtcagcaatataacagctatcccctcacgttcggtgctgggaccatgctggacctgaaacgggcggccgcatctactactaccaagccagtgctgcgaactccctcacctgtgcaccctaccgggacatctcagccccagagaccagaagattgtcggccccgtggctcagtgaaggggaccggattggacttcgcctgtgatatttacatctgggcacccttggccggaatctgcgtggcccttctgctgtccttgatcatcactctcatctgctacaatagtagaaggaacagactccttcaaagtgactacatgaacatgactccccggaggcctgggctcactcgaaagccttaccagccctacgcccctgccagagactttgcagcgtaccgccccagagcaaaattcagcaggagtgcagagactgctgccaacctgcaggaccccaaccagctctacaatgagctcaatctagggcgaagagaggaatatgacgtcttggagaagaagcgggctcgggatccagagatgggaggcaaacagcagaggaggaggaacccccaggaaggcgtatacaatgcactgcagaaagacaagatggcagaagcctacagtgagatcggcacaaaaggcgagaggcggagaggcaaggggcacgatggcctttaccagggtctcagcactgccaccaaggacacctatgatgccctgcatatgcagaccctggcccctcgctaa

SEQ ID NO: 38 - protein, 15 aa, synthetic construct
  REGION 1..15: note = Linker
GGGGSGGGGSGGGGS

SEQ ID NO: 39 - protein, 327 aa, synthetic construct
  REGION 1..327: note = IgG4-Fc
ASTKGPSVFPLAPCSRSTSESTAALGCLVKDYFPEPVTVSWNSGALTSGVHTFPAVLQSSGLYSLSSVVTVPSSSLGTKTYTCNVDHKPSNTKVDKRVESKYGPPCPSCPAPEFLGGPSVFLFPPKPKDTLMISRTPEVTCVVVDVSQEDPEVQFNWYVDGVEVHNAKTKPREEQFNSTYRVVSVLTVLHQDWLNGKEYKCKVSNKGLPSSIEKTISKAKGQPREPQVYTLPPSQEEMTKNQVSLTCLVKGFYPSDIAVEWESNGQPENNYKTTPPVLDSDGSFFLYSRLTVDKSRWQEGNVFSCSVMHEALHNHYTQKSLSLSLGK

SEQ ID NO: 40 - protein, 229 aa, synthetic construct
  REGION 1..229: note = Hinge-CH2-CH3
ESKYGPPCPPCPAPEFLGGPSVFLFPPKPKDTLMISRTPEVTCVVVDVSQEDPEVQFNWYVDGVEVHNAKTKPREEQFNSTYRVVSVLTVLHQDWLNGKEYKCKVSNKGLPSSIEKTISKAKGQPREPQVYTLPPSQEEMTKNQVSLTCLVKGFYPSDIAVEWESNGQPENNYKTTPPVLDSDGSFFLYSRLTVDKSRWQEGNVFSCSVMHEALHNHYTQKSLSLSLGK

SEQ ID NO: 41 - protein, 119 aa, synthetic construct
  REGION 1..119: note = Hinge-CH3
ESKYGPPCPPCPGQPREPQVYTLPPSQEEMTKNQVSLTCLVKGFYPSDIAVEWESNGQPENNYKTTPPVLDSDGSFFLYSRLTVDKSRWQEGNVFSCSVMHEALHNHYTQKSLSLSLGK

SEQ ID NO: 42 - protein, 12 aa, synthetic construct
  REGION 1..12: note = Hinge only
ESKYGPPCPPCP

SEQ ID NO: 43 - protein, 28 aa, Homo sapiens
MFWVLVVVGGVLACYSLLVTVAFIIFWV

SEQ ID NO: 44 - protein, 41 aa, synthetic construct
  REGION 1..41: note = cytoplasmic domain of CD28 with LL to GG substitution
RSKRSRGGHSDYMNMTPRRPGPTRKHYQPYAPPRDFAAYRS

SEQ ID NO: 45 - protein, 42 aa, Homo sapiens
KRGRKKLLYIFKQPFMRPVQTTQEEDGCSCRFPEEEEGGCEL

SEQ ID NO: 46 - protein, 112 aa, Homo sapiens
RVKFSRSADAPAYQQGQNQLYNELNLGRREEYDVLDKRRGRDPEMGGKPRRKNPQEGLYNELQKDKMAEAYSEIGMKGERRRGKGHDGLYQGLSTATKDTYDALHMQALPPR

SEQ ID NO: 47 - protein, 24 aa, synthetic construct
  REGION 1..24: note = T2A ribosomal skip element
LEGGGEGRGSLLTCGDVEENPGPR

SEQ ID NO: 48 - protein, 356 aa, synthetic construct
  REGION 1..356: note = tEGFR
MLLLVTSLLLCELPHPAFLLIPRKVCNGIGIGEFKDSLSINATNIKHFKNCTSISGDLHILPVAFRGDSFTHTPPLDPQELDILKTVKEITGFLLIQAWPENRTDLHAFENLEIIRGRTQHGQFSLAVVSLNITSLGLRSLKEISDGDVIISGNKNLCYANTINWKKLFGTSGQKTKIISNRGENSCKATGQVCHALCSPEGCWGPEPRDCVSCRNVSRGRECVDKCNLLEGEPREFVENSECIQCHPECLPQAMNITCTGRGPDNCIQCAHYIDGPHCVKTCPAGVMGENNTLVWKYADAGHVCHLCHPNCTYGCTGPGLEGCPTNGPKIPSIATGMVGALLLLLVVALGIGLFM

SEQ ID NO: 49 - protein, 8 aa, synthetic construct
  REGION 1..8: note = STREP TAG II
WSHPQFEK

SEQ ID NO: 50 - protein, 10 aa, synthetic construct
  REGION 1..10: note = Myc tag
EQKLISEEDL

SEQ ID NO: 51 - protein, 14 aa, synthetic construct
  REGION 1..14: note = V5 tag
GKPIPNPLLGLDST

SEQ ID NO: 52 - protein, 8 aa, synthetic construct
  REGION 1..8: note = FLAG tag
DYKDDDDK

SEQ ID NO: 53 - DNA, 20 bp, synthetic construct
  misc_feature 1..20: note = TRAC-Forward
  source 1..20: mol_type = other DNA
cccgtgtcattctctggact

SEQ ID NO: 54 - DNA, 20 bp, synthetic construct
  misc_feature 1..20: note = TRAC-Reverse
  source 1..20: mol_type = other DNA
atcacgagcagctggtttct

SEQ ID NO: 55 - DNA, 20 bp, synthetic construct
  misc_feature 1..20: note = Foxo13A Forward
  source 1..20: mol_type = other DNA
ggacagcctagaaagagcag

SEQ ID NO: 56 - DNA, 22 bp, synthetic construct
  misc_feature 1..22: note = Foxo13A Probe
  source 1..22: mol_type = other DNA
aggtcggcgtagctcagattgc

SEQ ID NO: 57 - DNA, 21 bp, synthetic construct
  misc_feature 1..21: note = Foxo13A Reverse
  source 1..21: mol_type = other DNA
ctcttgaccatccactcgtag